European Patent Application EP 4 477 746 A1, published December 18, 2024. Title: A method for determining the differentiation ability of cells in a culture medium, in the differentiation of pluripotent stem cells into neural cells in the midbrain floor plate region. Applicant: 住友ファーマ株式会社. The sequence listing filed with the application follows.

SEQUENCE LISTING (1 sequence)

SEQ ID NO: 1 - protein, 12 aa, synthetic construct
  REGION 1..12: note = L803-mts
  SITE 1: note = MISC_FEATURE - N-myristoyl glycine
  SITE 11: note = MISC_FEATURE - phosphorylated serine
  SITE 12: note = MISC_FEATURE - C-amidated proline
GKEAPPAPPQSP